European Patent Application EP 4 180 452 A1, published May 17, 2023. Title: FUSION PROTEIN COMPRISING GLUCAGON-LIKE PEPTIDE-1 AND IL-1 RECEPTOR ANTAGONIST AND USE THEREOF. Applicant: GI Innovation, Inc. The sequence listing filed with the application follows.

SEQUENCE LISTING (23 sequences)

SEQ ID NO: 1 - protein, 30 aa, Artificial Sequence
  hGLP-1
HAEGTFTSDVSSYLEGQAAKEFIAWLVKGR

SEQ ID NO: 2 - protein, 31 aa, Artificial Sequence
  hGLP-1 mt-1
HGEGTFTSDVSSYLEEQAAKEFIAWLVKGGG

SEQ ID NO: 3 - protein, 39 aa, Artificial Sequence
  hGLP-1 mt-2(exendin-4)
HGEGTFTSDLSKQMEEEAVRLFIEWLKNGGPSSGAPPPS

SEQ ID NO: 4 - protein, 31 aa, Artificial Sequence
  hGLP-1 mt-3(liraglutide)
HAEGTFTSDVSSYLEGQAAKEFIAWLVRGRG

SEQ ID NO: 5 - protein, 30 aa, Artificial Sequence
  NL028 hinge linker
GGGGSGGGGSGGGGSGGAESKYGPPCPPCP

SEQ ID NO: 6 - protein, 216 aa, Artificial Sequence
  hIgG4Fc
APEAAGGPSVFLFPPKPKDQLMISRTPEVTCVVVDVSQEDPEVQFNWYVDGVEVHNAKTKPREEQFNSTYRVVSVLTVLHQDWLNGKEYKCKVSNKGLPSSIEKTISKAKGQPREPQVYTLPPSQEEMTKNQVSLTCLVKGFYPSDIAVEWESNGQPENNYKTTPPVLDSDGSFFLYSRLTVDKSRWQEGNVFSCSVLHEALHNHYTQKSLSLSLG

SEQ ID NO: 7 - protein, 17 aa, Artificial Sequence
  (G4S)3GG linker
GGGGSGGGGSGGGGSGG

SEQ ID NO: 8 - protein, 152 aa, Artificial Sequence
  IL-1Ra
RPSGRKSSKMQAFRIWDVNQKTFYLRNNQLVAGYLQGPNVNLEEKIDVVPIEPHALFLGIHGGKMCLSCVKSGDETRLQLEAVNITDLSENRKQDKRFAFIRSDSGPTTSFESAACPGWFLCTAMEADQPVSLTNMPDEGVMVTKFYFQEDE

SEQ ID NO: 9 - protein, 19 aa, Artificial Sequence
  mIgG signal
MEWSWVFLFFLSVTTGVHS

SEQ ID NO: 10 - protein, 446 aa, Artificial Sequence
  GI-210B1(GLP-1-IgG4 Fc-IL-1Ra)
HGEGTFTSDVSSYLEEQAAKEFIAWLVKGGGGGGGSGGGGSGGGGSGGAESKYGPPCPPCPAPEAAGGPSVFLFPPKPKDQLMISRTPEVTCVVVDVSQEDPEVQFNWYVDGVEVHNAKTKPREEQFNSTYRVVSVLTVLHQDWLNGKEYKCKVSNKGLPSSIEKTISKAKGQPREPQVYTLPPSQEEMTKNQVSLTCLVKGFYPSDIAVEWESNGQPENNYKTTPPVLDSDGSFFLYSRLTVDKSRWQEGNVFSCSVLHEALHNHYTQKSLSLSLGGGGGSGGGGSGGGGSGGRPSGRKSSKMQAFRIWDVNQKTFYLRNNQLVAGYLQGPNVNLEEKIDVVPIEPHALFLGIHGGKMCLSCVKSGDETRLQLEAVNITDLSENRKQDKRFAFIRSDSGPTTSFESAACPGWFLCTAMEADQPVSLTNMPDEGVMVTKFYFQEDE

SEQ ID NO: 11 - DNA, 90 bp, Artificial Sequence
  hGLP-1
catgccgagggcacctttacctccgacgtgtcctcctacttggaggaacaggccgccaaagagtttatcgcctggctggtcaaaggtagg

SEQ ID NO: 12 - DNA, 93 bp, Artificial Sequence
  hGLP-1 mt-1
catggcgagggcacctttacctccgacgtgtcctcctacttggaggaacaggccgccaaagagtttatcgcctggctggtcaaaggtggcggc

SEQ ID NO: 13 - DNA, 90 bp, Artificial Sequence
  NL028 hinge linker
ggaggcggaggatccggtggtggtggatctggtggcggaggttctggcggagctgagtctaagtatggccctccttgtcctccatgtcct

SEQ ID NO: 14 - DNA, 648 bp, Artificial Sequence
  hIgG4Fc
gctccagaagctgctggcgggccctccgtgtttctgttccctccaaagcctaaggaccagctgatgatctctcggacccctgaagtgacctgcgtggtggtcgatgtgtcccaagaggaccctgaggtgcagttcaattggtacgtggacggcgtggaagtgcacaacgccaagaccaagcctagagaggaacagttcaactccacctacagagtggtgtccgtgctgaccgtgctgcaccaggattggctgaacggcaaagagtacaagtgcaaggtgtccaacaagggcctgccttccagcatcgaaaagaccatctccaaggccaagggccagcctagggaaccccaggtttacaccctgcctccaagccaagaggaaatgaccaagaaccaggtgtccctgacctgcctggtcaagggcttctacccttccgacattgccgtggaatgggagagcaatggccagcctgagaacaactacaagaccacacctcctgtgctggactccgacggctccttctttctgtactcccgcctgaccgtggacaagtccagatggcaagagggcaacgtgttctcctgctctgtgctgcacgaggccctgcacaatcactacacccagaagtccctcagcctgtcccttgga

SEQ ID NO: 15 - DNA, 51 bp, Artificial Sequence
  (G4S)3GG linker
ggtggtggcggctctggcggtggcggaagtggcggaggtggatccggaggt

SEQ ID NO: 16 - DNA, 456 bp, Artificial Sequence
  IL-1Ra
agaccttctggccggaagtcctctaagatgcaggccttcagaatctgggacgtgaaccagaaaaccttctacctgcggaacaaccagctcgtggccggctatctccagggacctaacgtgaacctggaagagaagatcgacgtggtgcccatcgagccccacgctctgtttttgggaatccacggcggcaagatgtgcctgtcctgtgtgaagtctggcgacgagacacggttgcagctggaagccgtgaacatcaccgacctgtccgagaaccggaagcaggacaagagattcgccttcatcagatccgacagcggccctaccacctccttcgagtctgctgcttgtccaggctggttcctgtgcaccgccatggaagctgaccagcctgtgtctctgaccaacatgcctgacgagggcgtgatggtcaccaagttctacttccaagaggatgag

SEQ ID NO: 17 - DNA, 57 bp, Artificial Sequence
  mIgG signal
atggaatggtcctgggtgttcctgttcttcctgtccgtgaccaccggcgtgcactct

SEQ ID NO: 18 - DNA, 1395 bp, Artificial Sequence
  Polynucleotides coding GI-210B1 with signal peptide
atggaatggtcctgggtgttcctgttcttcctgtccgtgaccaccggcgtgcactctcatggcgagggcacctttacctccgacgtgtcctcctacttggaggaacaggccgccaaagagtttatcgcctggctggtcaaaggtggcggcggaggcggaggatccggtggtggtggatctggtggcggaggttctggcggagctgagtctaagtatggccctccttgtcctccatgtcctgctccagaagctgctggcgggccctccgtgtttctgttccctccaaagcctaaggaccagctgatgatctctcggacccctgaagtgacctgcgtggtggtcgatgtgtcccaagaggaccctgaggtgcagttcaattggtacgtggacggcgtggaagtgcacaacgccaagaccaagcctagagaggaacagttcaactccacctacagagtggtgtccgtgctgaccgtgctgcaccaggattggctgaacggcaaagagtacaagtgcaaggtgtccaacaagggcctgccttccagcatcgaaaagaccatctccaaggccaagggccagcctagggaaccccaggtttacaccctgcctccaagccaagaggaaatgaccaagaaccaggtgtccctgacctgcctggtcaagggcttctacccttccgacattgccgtggaatgggagagcaatggccagcctgagaacaactacaagaccacacctcctgtgctggactccgacggctccttctttctgtactcccgcctgaccgtggacaagtccagatggcaagagggcaacgtgttctcctgctctgtgctgcacgaggccctgcacaatcactacacccagaagtccctcagcctgtcccttggaggtggtggcggctctggcggtggcggaagtggcggaggtggatccggaggtagaccttctggccggaagtcctctaagatgcaggccttcagaatctgggacgtgaaccagaaaaccttctacctgcggaacaaccagctcgtggccggctatctccagggacctaacgtgaacctggaagagaagatcgacgtggtgcccatcgagccccacgctctgtttttgggaatccacggcggcaagatgtgcctgtcctgtgtgaagtctggcgacgagacacggttgcagctggaagccgtgaacatcaccgacctgtccgagaaccggaagcaggacaagagattcgccttcatcagatccgacagcggccctaccacctccttcgagtctgctgcttgtccaggctggttcctgtgcaccgccatggaagctgaccagcctgtgtctctgaccaacatgcctgacgagggcgtgatggtcaccaagttctacttccaagaggatgag

SEQ ID NO: 19 - protein, 465 aa, Artificial Sequence
  GI-210B1 with signal peptide
MEWSWVFLFFLSVTTGVHSHGEGTFTSDVSSYLEEQAAKEFIAWLVKGGGGGGGSGGGGSGGGGSGGAESKYGPPCPPCPAPEAAGGPSVFLFPPKPKDQLMISRTPEVTCVVVDVSQEDPEVQFNWYVDGVEVHNAKTKPREEQFNSTYRVVSVLTVLHQDWLNGKEYKCKVSNKGLPSSIEKTISKAKGQPREPQVYTLPPSQEEMTKNQVSLTCLVKGFYPSDIAVEWESNGQPENNYKTTPPVLDSDGSFFLYSRLTVDKSRWQEGNVFSCSVLHEALHNHYTQKSLSLSLGGGGGSGGGGSGGGGSGGRPSGRKSSKMQAFRIWDVNQKTFYLRNNQLVAGYLQGPNVNLEEKIDVVPIEPHALFLGIHGGKMCLSCVKSGDETRLQLEAVNITDLSENRKQDKRFAFIRSDSGPTTSFESAACPGWFLCTAMEADQPVSLTNMPDEGVMVTKFYFQEDE

SEQ ID NO: 20 - DNA, 1338 bp, Artificial Sequence
  Polynucleotides coding GI-210B1
catggcgagggcacctttacctccgacgtgtcctcctacttggaggaacaggccgccaaagagtttatcgcctggctggtcaaaggtggcggcggaggcggaggatccggtggtggtggatctggtggcggaggttctggcggagctgagtctaagtatggccctccttgtcctccatgtcctgctccagaagctgctggcgggccctccgtgtttctgttccctccaaagcctaaggaccagctgatgatctctcggacccctgaagtgacctgcgtggtggtcgatgtgtcccaagaggaccctgaggtgcagttcaattggtacgtggacggcgtggaagtgcacaacgccaagaccaagcctagagaggaacagttcaactccacctacagagtggtgtccgtgctgaccgtgctgcaccaggattggctgaacggcaaagagtacaagtgcaaggtgtccaacaagggcctgccttccagcatcgaaaagaccatctccaaggccaagggccagcctagggaaccccaggtttacaccctgcctccaagccaagaggaaatgaccaagaaccaggtgtccctgacctgcctggtcaagggcttctacccttccgacattgccgtggaatgggagagcaatggccagcctgagaacaactacaagaccacacctcctgtgctggactccgacggctccttctttctgtactcccgcctgaccgtggacaagtccagatggcaagagggcaacgtgttctcctgctctgtgctgcacgaggccctgcacaatcactacacccagaagtccctcagcctgtcccttggaggtggtggcggctctggcggtggcggaagtggcggaggtggatccggaggtagaccttctggccggaagtcctctaagatgcaggccttcagaatctgggacgtgaaccagaaaaccttctacctgcggaacaaccagctcgtggccggctatctccagggacctaacgtgaacctggaagagaagatcgacgtggtgcccatcgagccccacgctctgtttttgggaatccacggcggcaagatgtgcctgtcctgtgtgaagtctggcgacgagacacggttgcagctggaagccgtgaacatcaccgacctgtccgagaaccggaagcaggacaagagattcgccttcatcagatccgacagcggccctaccacctccttcgagtctgctgcttgtccaggctggttcctgtgcaccgccatggaagctgaccagcctgtgtctctgaccaacatgcctgacgagggcgtgatggtcaccaagttctacttccaagaggatgag

SEQ ID NO: 21 - protein, 9 aa, Artificial Sequence
  Additional peptides
PSSGAPPPS

SEQ ID NO: 22 - protein, 277 aa, Artificial Sequence
  GLP-1-IgG4 Fc
HGEGTFTSDVSSYLEEQAAKEFIAWLVKGGGGGGGSGGGGSGGGGSGGAESKYGPPCPPCPAPEAAGGPSVFLFPPKPKDQLMISRTPEVTCVVVDVSQEDPEVQFNWYVDGVEVHNAKTKPREEQFNSTYRVVSVLTVLHQDWLNGKEYKCKVSNKGLPSSIEKTISKAKGQPREPQVYTLPPSQEEMTKNQVSLTCLVKGFYPSDIAVEWESNGQPENNYKTTPPVLDSDGSFFLYSRLTVDKSRWQEGNVFSCSVLHEALHNHYTQKSLSLSLG

SEQ ID NO: 23 - DNA, 831 bp, Artificial Sequence
  Polynucleotides coding GLP-1-IgG4 Fc
catggcgagggcacctttacctccgacgtgtcctcctacttggaggaacaggccgccaaagagtttatcgcctggctggtcaaaggtggcggcggaggcggaggatccggtggtggtggatctggtggcggaggttctggcggagctgagtctaagtatggccctccttgtcctccatgtcctgctccagaagctgctggcgggccctccgtgtttctgttccctccaaagcctaaggaccagctgatgatctctcggacccctgaagtgacctgcgtggtggtcgatgtgtcccaagaggaccctgaggtgcagttcaattggtacgtggacggcgtggaagtgcacaacgccaagaccaagcctagagaggaacagttcaactccacctacagagtggtgtccgtgctgaccgtgctgcaccaggattggctgaacggcaaagagtacaagtgcaaggtgtccaacaagggcctgccttccagcatcgaaaagaccatctccaaggccaagggccagcctagggaaccccaggtttacaccctgcctccaagccaagaggaaatgaccaagaaccaggtgtccctgacctgcctggtcaagggcttctacccttccgacattgccgtggaatgggagagcaatggccagcctgagaacaactacaagaccacacctcctgtgctggactccgacggctccttctttctgtactcccgcctgaccgtggacaagtccagatggcaagagggcaacgtgttctcctgctctgtgctgcacgaggccctgcacaatcactacacccagaagtccctcagcctgtcccttgga